European Patent Application EP 4 421 164 A1, published August 28, 2024. Title: Neurodegeneration and muscular atrophy model animal. Applicant: Tokyo Metropolitan Institute of Medical Science. The sequence listing filed with the application follows.

SEQUENCE LISTING (18 sequences)

SEQ ID NO: 1 - DNA, 20 bp, synthetic construct
  misc_feature 1..20: note = Synthetic DNA
  source 1..20: mol_type = other DNA
acttgcctgttatgtgtagg

SEQ ID NO: 2 - DNA, 20 bp, synthetic construct
  misc_feature 1..20: note = Synthetic DNA
  source 1..20: mol_type = other DNA
tgatgacatcaaggatgctc

SEQ ID NO: 3 - DNA, 20 bp, synthetic construct
  misc_feature 1..20: note = Synthetic DNA
  source 1..20: mol_type = other DNA
ccctggttcaattcccagta

SEQ ID NO: 4 - DNA, 20 bp, synthetic construct
  misc_feature 1..20: note = Synthetic DNA
  source 1..20: mol_type = other DNA
ggagtttgcatgaccacaga

SEQ ID NO: 5 - DNA, 21 bp, synthetic construct
  misc_feature 1..21: note = Synthetic DNA
  source 1..21: mol_type = other DNA
ccttcctgaagcagtagagca

SEQ ID NO: 6 - DNA, 20 bp, synthetic construct
  misc_feature 1..20: note = Synthetic DNA
  source 1..20: mol_type = other DNA
gccttattgtggaaggactg

SEQ ID NO: 7 - DNA, 27 bp, synthetic construct
  misc_feature 1..27: note = Synthetic DNA
  source 1..27: mol_type = other DNA
tgatagatccattcctatgactgtaga

SEQ ID NO: 8 - DNA, 27 bp, synthetic construct
  misc_feature 1..27: note = Synthetic DNA
  source 1..27: mol_type = other DNA
aagacattctttccagttaaagttgag

SEQ ID NO: 9 - DNA, 20 bp, synthetic construct
  misc_feature 1..20: note = Synthetic DNA
  source 1..20: mol_type = other DNA
tgccagcatctatgtggttc

SEQ ID NO: 10 - DNA, 20 bp, synthetic construct
  misc_feature 1..20: note = Synthetic DNA
  source 1..20: mol_type = other DNA
cacacactccttcccatcag

SEQ ID NO: 11 - DNA, 18 bp, synthetic construct
  misc_feature 1..18: note = Synthetic DNA
  source 1..18: mol_type = other DNA
ggagggggtggagctaga

SEQ ID NO: 12 - DNA, 19 bp, synthetic construct
  misc_feature 1..19: note = Synthetic DNA
  source 1..19: mol_type = other DNA
cgccacactctgctagtgc

SEQ ID NO: 13 - DNA, 20 bp, synthetic construct
  misc_feature 1..20: note = Synthetic DNA
  source 1..20: mol_type = other DNA
ggggagctgtgatgtgaagt

SEQ ID NO: 14 - DNA, 22 bp, synthetic construct
  misc_feature 1..22: note = Synthetic DNA
  source 1..22: mol_type = other DNA
ccaggaaataattctggctcat

SEQ ID NO: 15 - DNA, 20 bp, synthetic construct
  misc_feature 1..20: note = Synthetic DNA
  source 1..20: mol_type = other DNA
agtgaggaccggctactgtg

SEQ ID NO: 16 - DNA, 20 bp, synthetic construct
  misc_feature 1..20: note = Synthetic DNA
  source 1..20: mol_type = other DNA
gatcaaacgcttgcgaatct

SEQ ID NO: 17 - DNA, 22 bp, synthetic construct
  misc_feature 1..22: note = Synthetic DNA
  source 1..22: mol_type = other DNA
tgacatctacaagcaggagtgc

SEQ ID NO: 18 - DNA, 19 bp, synthetic construct
  misc_feature 1..19: note = Synthetic DNA
  source 1..19: mol_type = other DNA
tcgtcttcgtgttccttgc